European Patent Application EP 4 726 051 A1, published April 15, 2026. Title: Recombinant yeast, method for producing protein of interest, kit, and method for producing recombinant yeast. Applicant: FUJIFILM Corporation. Application WO. The sequence listing filed with the application follows.

SEQUENCE LISTING (19 sequences)

SEQ ID NO: 1 - DNA, 10511 bp, Ogataea parapolymorpha
  source 1..10511: mol_type = genomic DNA
gtattcccggaaagaactcgggatacggccggattattagctaaacgagccatgttagcaaaacggttggcgaggtttatttttttatttacatttcactgcaagtcgatcgaccgtgtcgcgactaatgaataatgaatatattatgaaatgtcaagattcaactagtctatcccaatctggctccgcaaacgcttcgactgtctcataaaacaaagaaaatattcaactatatacctttattaggctgtaaaatctaattgacctcgatcagtctaccctcatatggttgcagcttgcctgtgatgttgtttgcaatattagacaggagcagctttccttgagggattgggtactcgacttctctatcagtaaagttcaaaacaacagccatcttcttttggcctttgttgctggtcttggtgtagtagaaaacctcctggttatcgtagtcttgcacctcgaaacggccaaaagtcaacgtctcaggataaagctttctggtcttgatggcatttctgtaaaagttgagcacagagttagggtcatctttctgcgaagcaacgttgatgtctttgtagttgtcgttgattctcatccaaggcttaccaccgaaaccaccgttttcagaagagtcccactgaactggagtccttgcattgtctcttgccagcaaattgatgatcttcagcagctcggccttctcctcatcagagtgctcggtctcgttgaacgcgttccagtagttaatggtgttgatatccaaatactctgaaatatcccatttcggtgaaacatttgtcataccaatctcttgaccttggtacacaaacagagtgccggtcaaggttgtctgcaacagtgccagcatctttgcagatctgctccaaaacagtttgttggaggtgtttccgaaccttgtgacacagcgtggttggtcgtggttctcgataaaaacggtggaccatgcgtcattcagctcaccggtctcgtcatcaaagatgaattctgactggttgatgatggcatccttgaagtcggtcaagttgaagcctttgtatctaaaacggtcgctcttgtcggatccaacgtcaacagtgtcgaacaggaacatcatgttcatctccttttcttttgcagagacgtacttgagagcatctgccttggagcagtgaccaacttctccgacagtcatggcatcatacctggaagtcactttctcgtacatctctttgtggaactcgtgaatacgtggaccggagttgatgagtggaccagccggctggtatttctcacctgggaaggtgattggcgcatcctcaaaagtctggacttttgagtagaggccagcagtgtcgattctgaaaccagaaacgcccttctcgtaccaaaactcaagagcagatttgtaaatggcttcacgggtctctgggttctcccagttcaaatcaggctgagtctcagcaaacaggcgaaggtagtattgcttagtcttttcgtcataagcccatgcagaaccagagaaaaaggaaagccagttgttggcattgtccttccaaatgtaccaatctctctttggattgtctctgctagatctagactccttgaaccaagcgtgctcagacgaggtgtggttaataacgaggtccagaatcaatctcatgtctctcttcttgatctcggcaagcagtctgtccatgtcctccatagtgccaaattgagggttgatggcattgtagtcagaaatatcgtatcccatatcgtccaatggcgaagcatagtgcggagaaagccagatcacatcagtaccaagggatttgatatggtcgagctcggaagtgattccgtttaagtctccaataccgtctccgttggagtctttgaaggaagcaggccaaacttggtaaacaacggcggatttccaccaaggttcttgagactcgatagtcataaggaattaatattgtcaagagggataaaaaaattgtggaggcggagggtctttatatggcttgagcttactaaagacattctcatcactttagcgagcgcgacgctttggtatcctcctaacttcccgaaaataaaaagaggatttccgtttgcgtcatgggctccacctcctatgcacgtccataatagttatttgattgttatctgtaccccagacaagatcctgtttcagcgagtattaaatcacggcctaatttatttgagcgagaattaatttgcacatttaattctcgctgaaataactgccaacaattgagtctggggtacatgaatagaagtgacgtaattgacccccacgcttgctagccactgcggagtcacttgaaccacatgagagcccgtagggaagccagagcaatcaacgtcaaagggctcttaggaaacttgtataacccaagtgttcattacgacgctgcagagctctcacattatatgtagagtggtacggcagagtctgtagaacatacaaagctatcatgtcgcgtaatctgcacagtgcctgctttctattgcgatactcccgaagatatccctatccgcatacacggaactgtagttaatttgccgtggagtatcaatgtttgtccaacgcgccgaaactctttttgcggggctcttcttcatctaactcgtcctaagctggctcggggtatcgcataaacgtctgcgtgcattgccaagttgttttggtctgtgttgaaccttctttccaagccccatcccgaaccccggaaaattccccgattattatttccccgcaaatgcggcgtgccagaatctctcagccttgcgtcataatttagatttcgcaattatttcgtggagcaataggccgcgagcgtcctattgtgctgttggctcgaatctcatgcacaaaaatgaggatttgccagagtgtgttttccaaggcgtggccaaaacagagggtcaccagacaacagagctcaccataatacacagctttatggtcttacactaagtcctcctcctcaacaacgcggggctatacgtgtttgcagaattcttccatgcgtgatttgcaatggtgcttgcatactgcaacaatgcgtatggggtaattaaaacgagcactcgcgagcattcatcaaaggtaaaaagcattattctaagctctttctggaagcaaacttgggccgcgatcacgcaccaaaattcagccggattaagaatgggcaagcatctccccacgtcatatttgtgtggcattaggactatatatagttgatatattctcgacacactagtatccatcagcatgcctgagttcgtcgaaaacatcgagaagcctgaagaagtggaagtcattccagacatcacaaagaaaattaacactctttctgacagtgatgatggaagtggtgctttcaacgactacattgccagattcgtggagatttcgacgaatgcccagaataatgagcatcaagaaaaacacatgtcgctgaaggaaggtctgaaaactttcccgaaagctgcctgctggtcgattgtgctttccacagccatcatcatggaaggatacgataccatgctcttgaatagtttgtactcgatgcaatctttcgccaaaaaatacggccagtactacccggaaattgacgagtaccaggtccctgccaagtggcagacgtcgctttcgatgtcgacttatgtcggtgaaattgtcggactgtacattgcaggtcttgttgccgagaaatggggatacagacgtacgttgatatgcttcatggcagccgttgtgggtttaatcttcattcttttctttgcggtcgacgtgcagatgctgcttgccggcgagctgctctgtggtattgtctggggtgcattccagactcttacagtgtcatacgcctctgaagtctgtcccgttgtcctgagaatctaccttaccacttatgtcaatgcgtgctgggttatcggacagttaattgctgcttgtttgctgagaggcactatgaccctgaccaacgagtggtcatacaaaattcctttcgccgttcagtggatctggcctgtgccaatcatgattggaatctacctggccccggagtcgccctggtggctggttaaaaagaaccgggacgcagaagccaagagaagtatcatgagacttttgagtccaaacaccgaggtgccagacgttgctccgctagccgaggcaatgctgaacaaaatgcaactaaccatcaaggaagagtctgcgcgcacatccaatgtctcgtaccttgactgcttcaaacacggcaacttcagaagaacaaggattgcctccatgatctggctcatccagaatatcactggatctgtcttgatgggctattcgacctacttttacatccaggcaggacttgatagcggtatgtctttcactttctctatcatccaatatgcactgggtcttcttggaacaattgcctcgtggctgctgtcgcaaaaaatgggccgtttcgacatctatttcttgggtcttagcataaacacatgcatcctgataattgtcggaggtttgggcttctcttcatcgagcagtgcgtcttgggcaattggttcgttgctccttgtcttcacttttgtctacgactcatccatcggtcctatcacctactgtacggttgcagaaatcccttcgtcaacggtgcgtgccaagacagttgcccttgcaagaaactggtacaatctgtctcaaatcccgctctccattgtcactccatacatgctgaatccgactgcttggaactggaaagcaaaagcagcccttttatgggcaggcttgtctgtttgctcactgatctacatctggttcgagttcccagaaacaaaaggaagaacttatgctgaactggacatcctattcaaaaacggtaccagtgcccgtaagtttaagtccactcaggtggaaacattcaatcctgaggaaatgttaaaaaaaatgaataatgaggatattatacaggttgttgatggcgacctggatgccggtgcggccactgctaaagtttaaaagttgaaatgtatagtttcagttctgcgatgttattattttacaattgaatatgctatctcgaatgattttttgtaatagccgtagatgtctttattattgcatttaagggttcaaaattattcatgtgagcgttttattttacgggacaataagattttgggcgagacttccccacaaattgaataatgtgcaatatttttaagaactaaatttactggagacaatttctatgcctctcagtacacgtgcaaaaccacaaacgcctggccaaaagtcccattctaaaaggccgtatatcaggccttgtgacgcgtgcgcgttcaaaagagtacgttgcgatgctgagttcaagttggatcgcagatgcaccaactgtttagttcatggaattgagtgtacgaataacagagtcaagcagagatctggacccagaaaaatacataaaaaaactgaagaggctattaaaagcctggtagaaggaagtggcgcgttcagcaatcttcgattagccactccggcccacaacatatgtggtattatcaatcctgccacctgcgagaagagctcaatatcgcttagtgagattcgaccgtacctcagaatttataaatcccgatactatgcactctggccagtcctgtctgttgatgactgtctgaatattcttaatgaaagctcagttcacataaacgatagcgcatttttcatgctcaatgccaacaatgcgtcgttgtacgctctttcatgcgccttgtgcgctgtaattgcaagacacaccaccttctggtccctggaagaatttgatacaatggctcatttaggactcaaaagctgccctccgccagaaacttatgtaagggaggcagagcgagctatctacatgtttgaccttgacgggatactcacagaagaccaggttttaactaacttctttctgcatatatatttttcatcccttgacgaggacaacctgcaggaattggtctatctcagacaggcaatcagctgcgcacaaatgcttcaccttcgagataacgaagttttgggagaatcaccaaaagatacatcacacagatttaaaaaaatttactacttacttctcatcacagagaggtatgtctcgttcaaaaaacaactaccagtgatattagagccaacaatgccacttccaagtttggaagatgatgaagccccggatctgctacctggatttatcgaacttgcgcaagtattcagtgttcctgattgcgctttctttaacaagtactcgctccgtggcacgacagctgcacttgatcctttcagcgagagctttgacctaatgttcaaaaacgaatggatccaagacgtgcaaaccaagctctctaggtcggtcgttcaggtgcgcaaccagtctcaaaaggtcaatatattaatttctcgaacatggttgcaatcaattgcttggttaatggccaaagatcgacttcttctatcgcctacgagtgatcaagccaatttctttgatccaaggtatcctattcatatcgcgaaagactttctgatacagactaaagacatgccgtacgaggcatttgaaacaaacggtagtggtgtcatcgtgaaactaagcgaagtcgccaacgccttgcaaaccttcatccgattggctccaggatcgcccgaaacagctttagcattagacgagcttgcatatatccacggtattatcatgcggcagaactccaacagctcgctcgggcctcttatacaccctatcactgaaactttggaatctcgcaggttcggattttatcgaaatggctgcgacatttcttatccaaaaatagagtctgcagattatgaagagaacgaaaatgaccatacacccgaaatcattgcctccatgccggagaacttgaatttgacacctcttttgagcgagttcgaatttccgaggtgaacaagtattatctgctcacgtgtttggtgcattttgcaactagcgacaaatttcactggcatattagtatatcatcaaatcattaggattgctattttgtgtccactaaggcgctccaggtgcgtggaatggtgcagtattaggccctagctgtccgagaaaaaaggaagctacaccctttgatgtagtgggctctttgtgtgttgtgagaggattaaattggccagatgacactctttccaaagatgcaaataacgaggaagaaacatccagccggatgccagatgtctgtctgtgttgcaaattcgctcttgatccggaaaaagagttattgaaaagggcactgtcctgtctcgtattgcagcgtacgagtgaacctgagcgtgtcaatgcaggttcataagaagaaaattcagaagacagattgtgacatatttctcgcaagccattcactttccaagattctaggagcttagagatcttggtgaacagggctcggggcaagtccattccagctttgtacttcaacaccatgtcgaatacggcacccatgcgttcgtaggctagctcggtggttgctgggtcaacatagcttttgatcagaatgtaaagagagtctgctatctccagtaatttcattgatatgtcgggtccgttgcatctaaaggcatgatcagggaggttttgtagactgctgagaagctcatttgcaacttttagaggaaagttaatcttgaaacattcgtgttcgaccgcaatgctctcatcagaactaattagaaaattcgcagacgcaattaaccagcccaaagactggagccaggcttttgagacaataacattcactttttgagcacttgttgcaattttatccacatcaattctaatttggagcttctgttggagctcaaggagccacagcctcttcaactctgtggatccgttcaaggtaaaatcctgaaacaagttggtctctggaatctggaacatgttgtgagtgcgccctgtctcgagcactttagtatgaagctcaacatagaattgcttatccgttgcactgaaaattgcacacagagtggtgaacccgtaaagtgaatttgaggatttttcgaaatctgcttcagggagtggaattgaaggttcaagaagaacgggcaaattagttttaaagctgacaaacctttcggttaccacgagcaaatagtagatttttttctgcctatgagcctcaacgggtgacaaatgaagcagtgactgtggttcgtgcatttttaagatatctgcaagagaaacagcttcacggaggtaaataagacctttgtgctgttggccaggcgcaatagcatagtatttatgtaggaagaaggatgtcagaaggagatcaatatttggtgtgcttttcagtctatactcataaattatcctccttgcctcttgagcatataagccagcatttttgagatcgctcctggctggagtgtatgtgacgaaactgtgatattgtgcgatcgtagcgcacaatgcgcaacaaagagcatattcttgggcattgtcctcggcgatggtgatacgaaaatcatctaaaacattcgctagttgaaatacctgctccacattctttaaggggcttgaacgtgtcaaaattgaaactgtactttgaattgatactaccggccagatatcgtaaaaattcgaatgatatatctcaaggtaagggataatttgtttcaaagaaaatgcgcacacatgagcaggtagtgtagactgagcatagatttcgtcgttgagatcctctgtgtttttgactgttctagtacttttctttggaccggatttatgcctcacgcggaggttggtacatggaactttatgagtgagacagttcgagcaaataccaccggtgcatgaatctatatcgcacttcacacggcggatggcgcatgcgtcacagggtctcggccgttgtcgttttttggtggacggctgcgacatctcggtatttagataagccagcttgtacttgtatccaaaatgtggggctaaaggggagtgtatgatttttaatgatatcggtgaatgtccagaaatttggtaaatcgcacaccaaacttcaacgatggactagcgtgctaaactgatattctaccaaacaaccgtttgagtaattctgaccatgacagaggtcttgtgtatatattttaagccccgtcgatcgaccgcatcgcgactccataaaaaaattcatttcacgcgttattattatcgtatgaatatggatcccctaaacgtgaaagtgcaacagaaacttaaggagctcgaaagccttcagcagataagagacttgacgaaacacctgaatgtttcactggaagaatttgctggccaaatagaacttctgggtgaggaagcaggatgcatcgaaaccgtgacgcaaaactggatgagaatcatcagagcagtgagcctagcctctaactctttgtcgaactacaaggaagaggactatgaaacggatagaccaatgacggagcgccttgtgagatgcaagatagacgagagtcaaaaaatcatcaccaaaaattgacttacttcaatctatctaaccattgttctaaattgatcttgttgttcagttccgacaacagatcgttctccttcagcaaatcgtcacgaaggcctttatcagcctcgagataattaatatcgtccggatctaacattaagtcctgaactttagagggaagttctattttgagcgtcgataacccggtcatcattttgaagtattcattagtatgcacgtcagaaccattcaaaagcccatcccaatcagttgtcaaaaacagccttttccatatcaaggtttccaagatttcgtgatagtgcgaataaccactcaggttacttatcactcttgacggattggagtgtttgatgacagtcaacaatttgaacaagttggcgaaattgttgtgactgaattcatcaaacgtcactaatgtcagtagctggaccatctcaaacaatcccagctgttgctgcttatccatctttgccacaatatcgccgatctgactttcaaaatgtgtaaacttgttatcaaccaagtatcttgagtcttgtatgaatccatctttagtttttgaatcaattaatctcgcataattcaattgaagctcaatcatttgcaagtgtatttctatctcatccaacagattgtcgtgatcctcattcaaagctatcagtgaaagtttggcaatattcagttcgaactttttcttttcaatttcctccgactctgcagtggaaacatatgcaatcagcttttctgctgccttgaaatactcatcgttttccacgtcaagtatccaggcaaatttatagttgttgatgcttgaattcaaaaacatgcgcacgtaatctggatattgagggatgtaattgaggattagccgaatctttctggttctagcatagaatccaaaaagcacttctgcaaaacggtatccataccgctggaaacattcc

SEQ ID NO: 2 - DNA, 5978 bp, synthetic construct
  misc_feature 1..5978: note = Description of Artificial Sequence: recombinant DNA
  source 1..5978: mol_type = other DNA
caaatcaactgagaaaaatggtattcccggaaagaactcgggatacggccggattattagctaaacgagccatgttagcaaaacggttggcgaggtttatttttttatttacatttcactgcaagtcgatcgaccgtgtcgcgactaatgaataatgaatatattatgaaatgtcaagattcaactagtctatcccaatctggctccgcaaacgcttcgactgtctcataaaacaaagaaaatattcaactatatacctttattaggctgtaaaatctaattgacctcgatcagtctaccctcatatggttgcagcttgcctgtgatgttgtttgcaatattagacaggagcagctttccttgagggattgggtactcgacttctctatcagtaaagttcaaaacaacagccatcttcttttggcctttgttgctggtcttggtgtagtagaaaacctcctggttatcgtagtcttgcacctcgaaacggccaaaagtcaacgtctcaggataaagctttctggtcttgatggcatttctgtaaaagttgagcacagagttagggtcatctttctgcgaagcaacgttgatgtctttgtagttgtcgttgattctcatccaaggcttaccaccgaaaccaccgttttcagaagagtcccactgaactggagtccttgcattgtctcttgccagcaaattgatgatcttcagcagctcggccttctcctcatcagagtgctcggtctcgttgaacgcgttccagtagttaatggtgttgatatccaaatactctgaaatatcccatttcggtgaaacatttgtcataccaatctcttgaccttggtacacaaacagagtgccggtcaaggttgtctgcaacagtgccagcatctttgcagatctgctccaaaacagtttgttggaggtgtttccgaaccttgtgacacagcgtggttggtcgtggttctcgataaaaacggtggaccatgcgtcattcagctcaccggtctcgtcatcaaagatgaattctgactggttgatgatggcatccttgaagtcggtcaagttgaagcctttgtatctaaaacggtcgctcttgtcggatccaacgtcaacagtgtcgaacaggaacatcatgttcatctccttttcttttgcagagacgtacttgagagcatctgccttggagcagtgaccaacttctccgacagtcatggcatcatacctggaagtcactttctcgtacatctctttgtggaactcgtgaatacgtggaccggagttgatgagtggaccagccggctggtatttctcacctgggaaggtgattggcgcatcctcaaaagtctggacttttgagtagaggccagcagtgtcgattctgaaaccagaaacgcccttctcgtaccaaaactcaagagcagatttgtaaatggcttcacgggtctctgggttctcccagttcaaatcaggctgagtctcagcaaacaggcgaaggtagtattgcttagtcttttcgtcataagcccatgcagaaccagagaaaaaggaaagccagttgttggcattgtccttccaaatgtaccaatctctctttggattgtctctgctagatctagactccttgaaccaagcgtgctcagacgaggtgtggttaataacgaggtccagaatcaatctcatgtctctcttcttgatctcggcaagcagtctgtccatgtcctccatagtgccaaattgagggttgatggcattgtagtcagaaatatcgtatcccatatcgtccaatggcgaagcatagtgcggagaaagccagatcacatcagtaccaagggatttgatatggtcgagctcggaagtgattccgtttaagtctccaataccgtctccgttggagtctttgaaggaagcaggccaaacttggtaaacaacggcggatttccaccaaggttcttgagactcgatagtcataaggaattaatattgtcaagagggataaaaaaattgtggaggcggagggtctttatatggcttgagcttactaaagacattctcatcactttagcgagcgcgacgctttggtatcctcctaacttcccgaaaataaaaagaggatttccgtttgcgtcatgggctccacctcctatgcacgtccataatagttatttgattgttatctgtaccccagacaagatcctgtttcagcgagtattaaatcacggcctaatttatttgagcgagaattaatttgcacatttaattctcgctgaaataactgccaacaattgagtctggggtacatgaatagaagtgacgtaattgacccccacgcttgctagccactgcggagtcacttgaaccacatgagagcccgtagggaagccagagcaatcaacgtcaaagggctcttaggaaacttgtataacccaagtgttcattacgacgctgcagagctctcacattatatgtagagtggtacggcagagtctgtagaacatacaaagctatcatgtcgcgtaatctgcacagtgcctgctttctattgcgatactcccgaagatatccctatccgcatacacggaactgtagttaatttgccgtggagtatcaatgtttgtccaacgcgccgaaactctttttgcggggctcttcttcatctaactcgtcctaagctggctcggggtatcgcataaacgtctgcgtgcattgccaagttgttttggtctgtgttgaaccttctttccaagccccatcccgaaccccggaaaattccccgattattatttccccgcaaatgcggcgtgccagaatctctcagccttgcgtcataatttagatttcgcaattatttcgtggagcaataggccgcgagcgtcctattgtgctgttggctcgaatctcatgcacaaaaatgaggatttgccagagtgtgttttccaaggcgtggccaaaacagagggtcaccagacaacagagctcaccataatacacagctttatggtcttacactaagtcctcctcctcaacaacgcggggctatacgtgtttgcagaattcttccatgcgtgatttgcaatggtgcttgcatactgcaacaatgcgtatggggtaattaaaacgagcactcgcgagcattcatcaaaggtaaaaagcattattctaagctctttctggaagcaaacttgggccgcgatcacgcaccaaaattcagccggattaagaatgggcaagcatctccccacgtcatatttgtgtggcattaggactatatatagttgatatattctcgacacactagtatccatcagcatgcctgagttcgtcgaaaacatcgagaagcctgaagaagtggaagtcattccagacatcacaaagaaaattaacactctttctgacagtgatgatggaagtggtgctttcaacgactacattgccagattcgtggagatttcgacgaatgcccagaataatgagcatcaagaaaaacacatgtcgctgaaggaaggtctgaaaactttcccgaaagctgcctgctggtcgattgtgctttccacagccatcatcatggaaggatacgataccatgctcttgaatagtttgtactcgatgcaatctttcgccaaaaaatacggccagtactacccggaaattgacgagtaccaggtccctgccaagtggcagacgtcgctttcgatgtcgacttatgtcggtgaaattgtcggactgtacattgcaggtcttgttgccgagaaatggggatacagacgtacgttgatatgcttcatggcagccgttgtgggtttaatcttcattcttttctttgcggtcgacgtgcagatgctgcttgccggcgagctgctctgtggtattgtctggggtgcattccagactcttacagtgtcatacgcctctgaagtctgtcccgttgtcctgagaatctaccttaccacttatgtcaatgcgtgctgggttatcggacagttaattgctgcttgtttgctgagaggcactatgaccctgaccaacgagtggtcatacaaaattcctttcgccgttcagtggatctggcctgtgccaatcatgattggaatctacctggccccggagtcgccctggtggctggttaaaaagaaccgggacgcagaagccaagagaagtatcatgagacttttgagtccaaacaccgaggtgccagacgttgctccgctagccgaggcaatgctgaacaaaatgcaactaaccatcaaggaagagtctgcgcgcacatccaatgtctcgtaccttgactgcttcaaacacggcaacttcagaagaacaaggattgcctccatgatctggctcatccagaatatcactggatctgtcttgatgggctattcgacctacttttacatccaggcaggacttgatagcggtatgtctttcactttctctatcatccaatatgcactgggtcttcttggaacaattgcctcgtggctgctgtcgcaaaaaatgggccgtttcgacatctatttcttgggtcttagcataaacacatgcatcctgataattgtcggaggtttgggcttctcttcatcgagcagtgcgtcttgggcaattggttcgttgctccttgtcttcacttttgtctacgactcatccatcggtcctatcacctactgtacggttgcagaaatcccttcgtcaacggtgcgtgccaagacagttgcccttgcaagaaactggtacaatctgtctcaaatcccgctctccattgtcactccatacatgctgaatccgactgcttggaactggaaagcaaaagcagcccttttatgggcaggcttgtctgtttgctcactgatctacatctggttcgagttcccagaaacaaaaggaagaacttatgctgaactggacatcctattcaaaaacggtaccagtgcccgtaagtttaagtccactcaggtggaaacattcaatcctgaggaaatgttaaaaaaaatgaataatgaggatattatacaggttgttgatggcgacctggatgccggtgcggccactgctaaagtttaaaagttgaaatgtatagtttcagttctgcgatgttattattttacaattgaatatgctatctcgaatgattttttgtaatagccgtagatgtctttattattgcatttaagggttcaaaattattcatgtgagcgttttattttacgggacaataagattttgggcgagacttccccacaaattgaataatgtgcaatatttttaagaactaaatttactggagacaatttctatgcctctcagtacacgtgcaaaaccacaaacgcctggccaaaagtcccattctaaaaggccgtatatcaggccttgtgacgcgtgcgcgttcaaaagagtacgttgcgatgctgagttcaagttggatcgcagatgcaccaactgtttagttcatggaattgagtgtacgaataacagagtcaagcagagatctggacccagaaaaatacataaaaaaactgaagaggctattaaaagcctggtagaaggaagtggcgcgttcagcaatcttcgattagccactccggcccacaacatatgtggtattatcaatcctgccacctgcgagaagagctcaatatcgcttagtgagattcgaccgtacctcagaatttataaatcccgatactatgcactctggccagtcctgtctgttgatgactgtctgaatattcttaatgaaagctcagttcacataaacgatagcgcatttttcatgctcaatgccaacaatgcgtcgttgtacgctctttcatgcgccttgtgcgctgtaattgcaagacacaccaccttctggtccctggaagaatttgatacaatggctcatttaggactcaaaagctgccctccgccagaaacttatgtaagggaggcagagcgagctatctacatgtttgaccttgacgggatactcacagaagaccagg

SEQ ID NO: 3 - DNA, 1021 bp, synthetic construct
  misc_feature 1..1021: note = Description of Artificial Sequence: recombinant DNA
  source 1..1021: mol_type = other DNA
ttgtcagcttaaaggactccatttcctaaaatttcaagcagtcctctcaactaaatttttttccattcctctgcacccagccctcttcatcaaccgtccagccttctcaaaagtccaatgtaagtagcctgcaaattcaggttacaacccctcaattttccatccaagggcgatccttacaaagttaatatcgaacagcagagactaagcgagtcatcatcaccacccaacgatggtgaaaaactttaagcatagattgatggagggtgtatggcacttggcggctgcattagagtttgaaactatggggtaatacatcacatccggaactgatccgactccgagatcatatgcaaagcacgtgatgtaccccgtaaactgctcggattatcgttgcaattcatcgtcttaaacagtacaagaaactttattcatgggtcattggactctgatgaggggcacatttccccaatgattttttgggaaagaaagccgtaagaggacagttaagcgaaagagacaagacaacgaacagcaaaagtgacagctgtcagctacctagtggacagttgggagtttccaattggttggttttgaatttttacccatgttgagttgtccttgcttctccttgcaaacaatgcaagttgataagacatcaccttccaagataggctatttttgtcgcataaatttttgtctcggagtgaaaaccccttttatgtgaacagattacagaagcgtcctacccttcaccggttgagatggggagaaaattaagcgatgaggagacgattattggtataaaagaagcaaccaaaatcccttattgtccttttctgatcagcatcaaagaatattgtcttaaaacgggcttttaactacattgttcttacacattgcaaacctcttccttctatttcggatcaactgtattgactacattgatcttttttaacgaagtttacgacttactaaatccccacaaacaaatcaactgagaaaaatggtattcccggaa

SEQ ID NO: 4 - DNA, 5733 bp, synthetic construct
  misc_feature 1..5733: note = Description of Artificial Sequence: recombinant DNA
  source 1..5733: mol_type = other DNA
tgggcaggcttgtctgtttgctcactgatctacatctggttcgagttcccagaaacaaaaggaagaacttatgctgaactggacatcctattcaaaaacggtaccagtgcccgtaagtttaagtccactcaggtggaaacattcaatcctgaggaaatgttaaaaaaaatgaataatgaggatattatacaggttgttgatggcgacctggatgccggtgcggccactgctaaagtttaaaagttgaaatgtatagtttcagttctgcgatgttattattttacaattgaatatgctatctcgaatgattttttgtaatagccgtagatgtctttattattgcatttaagggttcaaaattattcatgtgagcgttttattttacgggacaataagattttgggcgagacttccccacaaattgaataatgtgcaatatttttaagaactaaatttactggagacaatttctatgcctctcagtacacgtgcaaaaccacaaacgcctggccaaaagtcccattctaaaaggccgtatatcaggccttgtgacgcgtgcgcgttcaaaagagtacgttgcgatgctgagttcaagttggatcgcagatgcaccaactgtttagttcatggaattgagtgtacgaataacagagtcaagcagagatctggacccagaaaaatacataaaaaaactgaagaggctattaaaagcctggtagaaggaagtggcgcgttcagcaatcttcgattagccactccggcccacaacatatgtggtattatcaatcctgccacctgcgagaagagctcaatatcgcttagtgagattcgaccgtacctcagaatttataaatcccgatactatgcactctggccagtcctgtctgttgatgactgtctgaatattcttaatgaaagctcagttcacataaacgatagcgcatttttcatgctcaatgccaacaatgcgtcgttgtacgctctttcatgcgccttgtgcgctgtaattgcaagacacaccaccttctggtccctggaagaatttgatacaatggctcatttaggactcaaaagctgccctccgccagaaacttatgtaagggaggcagagcgagctatctacatgtttgaccttgacgggatactcacagaagaccaggttttaactaacttctttctgcatatatatttttcatcccttgacgaggacaacctgcaggaattggtctatctcagacaggcaatcagctgcgcacaaatgcttcaccttcgagataacgaagttttgggagaatcaccaaaagatacatcacacagatttaaaaaaatttactacttacttctcatcacagagaggtatgtctcgttcaaaaaacaactaccagtgatattagagccaacaatgccacttccaagtttggaagatgatgaagccccggatctgctacctggatttatcgaacttgcgcaagtattcagtgttcctgattgcgctttctttaacaagtactcgctccgtggcacgacagctgcacttgatcctttcagcgagagctttgacctaatgttcaaaaacgaatggatccaagacgtgcaaaccaagctctctaggtcggtcgttcaggtgcgcaaccagtctcaaaaggtcaatatattaatttctcgaacatggttgcaatcaattgcttggttaatggccaaagatcgacttcttctatcgcctacgagtgatcaagccaatttctttgatccaaggtatcctattcatatcgcgaaagactttctgatacagactaaagacatgccgtacgaggcatttgaaacaaacggtagtggtgtcatcgtgaaactaagcgaagtcgccaacgccttgcaaaccttcatccgattggctccaggatcgcccgaaacagctttagcattagacgagcttgcatatatccacggtattatcatgcggcagaactccaacagctcgctcgggcctcttatacaccctatcactgaaactttggaatctcgcaggttcggattttatcgaaatggctgcgacatttcttatccaaaaatagagtctgcagattatgaagagaacgaaaatgaccatacacccgaaatcattgcctccatgccggagaacttgaatttgacacctcttttgagcgagttcgaatttccgaggtgaacaagtattatctgctcacgtgtttggtgcattttgcaactagcgacaaatttcactggcatattagtatatcatcaaatcattaggattgctattttgtgtccactaaggcgctccaggtgcgtggaatggtgcagtattaggccctagctgtccgagaaaaaaggaagctacaccctttgatgtagtgggctctttgtgtgttgtgagaggattaaattggccagatgacactctttccaaagatgcaaataacgaggaagaaacatccagccggatgccagatgtctgtctgtgttgcaaattcgctcttgatccggaaaaagagttattgaaaagggcactgtcctgtctcgtattgcagcgtacgagtgaacctgagcgtgtcaatgcaggttcataagaagaaaattcagaagacagattgtgacatatttctcgcaagccattcactttccaagattctaggagcttagagatcttggtgaacagggctcggggcaagtccattccagctttgtacttcaacaccatgtcgaatacggcacccatgcgttcgtaggctagctcggtggttgctgggtcaacatagcttttgatcagaatgtaaagagagtctgctatctccagtaatttcattgatatgtcgggtccgttgcatctaaaggcatgatcagggaggttttgtagactgctgagaagctcatttgcaacttttagaggaaagttaatcttgaaacattcgtgttcgaccgcaatgctctcatcagaactaattagaaaattcgcagacgcaattaaccagcccaaagactggagccaggcttttgagacaataacattcactttttgagcacttgttgcaattttatccacatcaattctaatttggagcttctgttggagctcaaggagccacagcctcttcaactctgtggatccgttcaaggtaaaatcctgaaacaagttggtctctggaatctggaacatgttgtgagtgcgccctgtctcgagcactttagtatgaagctcaacatagaattgcttatccgttgcactgaaaattgcacacagagtggtgaacccgtaaagtgaatttgaggatttttcgaaatctgcttcagggagtggaattgaaggttcaagaagaacgggcaaattagttttaaagctgacaaacctttcggttaccacgagcaaatagtagatttttttctgcctatgagcctcaacgggtgacaaatgaagcagtgactgtggttcgtgcatttttaagatatctgcaagagaaacagcttcacggaggtaaataagacctttgtgctgttggccaggcgcaatagcatagtatttatgtaggaagaaggatgtcagaaggagatcaatatttggtgtgcttttcagtctatactcataaattatcctccttgcctcttgagcatataagccagcatttttgagatcgctcctggctggagtgtatgtgacgaaactgtgatattgtgcgatcgtagcgcacaatgcgcaacaaagagcatattcttgggcattgtcctcggcgatggtgatacgaaaatcatctaaaacattcgctagttgaaatacctgctccacattctttaaggggcttgaacgtgtcaaaattgaaactgtactttgaattgatactaccggccagatatcgtaaaaattcgaatgatatatctcaaggtaagggataatttgtttcaaagaaaatgcgcacacatgagcaggtagtgtagactgagcatagatttcgtcgttgagatcctctgtgtttttgactgttctagtacttttctttggaccggatttatgcctcacgcggaggttggtacatggaactttatgagtgagacagttcgagcaaataccaccggtgcatgaatctatatcgcacttcacacggcggatggcgcatgcgtcacagggtctcggccgttgtcgttttttggtggacggctgcgacatctcggtatttagataagccagcttgtacttgtatccaaaatgtggggctaaaggggagtgtatgatttttaatgatatcggtgaatgtccagaaatttggtaaatcgcacaccaaacttcaacgatggactagcgtgctaaactgatattctaccaaacaaccgtttgagtaattctgaccatgacagaggtcttgtgtatatattttaagccccgtcgatcgaccgcatcgcgactccataaaaaaattcatttcacgcgttattattatcgtatgaatatggatcccctaaacgtgaaagtgcaacagaaacttaaggagctcgaaagccttcagcagataagagacttgacgaaacacctgaatgtttcactggaagaatttgctggccaaatagaacttctgggtgaggaagcaggatgcatcgaaaccgtgacgcaaaactggatgagaatcatcagagcagtgagcctagcctctaactctttgtcgaactacaaggaagaggactatgaaacggatagaccaatgacggagcgccttgtgagatgcaagatagacgagagtcaaaaaatcatcaccaaaaattgacttacttcaatctatctaaccattgttctaaattgatcttgttgttcagttccgacaacagatcgttctccttcagcaaatcgtcacgaaggcctttatcagcctcgagataattaatatcgtccggatctaacattaagtcctgaactttagagggaagttctattttgagcgtcgataacccggtcatcattttgaagtattcattagtatgcacgtcagaaccattcaaaagcccatcccaatcagttgtcaaaaacagccttttccatatcaaggtttccaagatttcgtgatagtgcgaataaccactcaggttacttatcactcttgacggattggagtgtttgatgacagtcaacaatttgaacaagttggcgaaattgttgtgactgaattcatcaaacgtcactaatgtcagtagctggaccatctcaaacaatcccagctgttgctgcttatccatctttgccacaatatcgccgatctgactttcaaaatgtgtaaacttgttatcaaccaagtatcttgagtcttgtatgaatccatctttagtttttgaatcaattaatctcgcataattcaattgaagctcaatcatttgcaagtgtatttctatctcatccaacagattgtcgtgatcctcattcaaagctatcagtgaaagtttggcaatattcagttcgaactttttcttttcaatttcctccgactctgcagtggaaacatatgcaatcagcttttctgctgccttgaaatactcatcgttttccacgtcaagtatccaggcaaatttatagttgttgatgcttgaattcaaaaacatgcgcacgtaatctggatattgagggatgtaattgaggattagccgaatctttctggttctagcatagaatccaaaaagcacttctgcaaaacggtatccataccgctggaaacattcctagtttatgttgtatctatg

SEQ ID NO: 5 - DNA, 1000 bp, synthetic construct
  misc_feature 1..1000: note = Description of Artificial Sequence: recombinant DNA
  source 1..1000: mol_type = other DNA
cataccgctggaaacattcctagtttatgttgtatctatgaatatttttttacatggtggatttgttccaatctagttgttagttatttgtcgttatagtcactaatacagttaccatcggaatcttttcatttctttttatacgtacgtatatgtactagatgaagaatgcgacaaggccgaccaacagcaatggtgcttggtaccaaagtttggaaggtgctaccgaattggccgatgatattgaagtggagttgtcattctcctcattggttgctccagtagtggtaaaattaacggggatatcttcggtggaagtgtcaatatcaccgttccaacaataattctcaaaacatcttctacattgctctgtttgtgttgcattggatctctcctgctgtctacgaatgattgcacatccaacacaagtacgccattcttcatcaatagtcatgttcaaacgagacgacacttcaaaaccgttttggatcattcctctcttctcggattcagagtagtctaacttgaaagttgaagtgttactccaatacgagaaaggtctattggccagataaacaaccaggggaggaatgtgatccgtgccttcaacaatgtctgtcaaatttctagcatcacaaccaaagaaggttggcttactcgaaagattcaagtttaggaaagtggtggtatcaggtacataagggaacgttgttccatttgcttgagaagaaaactgtctcatgtaggtgttgactaatgatgaaccgtttggccaagagaggtcagtgtctgcactgttgtcaaacgcaaagatgatatcaacgtcacgctccttttgaagtagaggctgcagagggacgttttggttatcctctccaccatcaaccaagtaaagggtgtcattttccgcaatggcacctactcctgcatacgtacttttgtagaaagggttgggggaatagatagcaatgtcgtcttcgtcttcgctaagtccagtcag

SEQ ID NO: 6 - DNA, 20 bp, synthetic construct
  misc_feature 1..20: note = Description of Artificial Sequence: primer
  source 1..20: mol_type = other DNA
ttgtcagcttaaaggactcc

SEQ ID NO: 7 - DNA, 40 bp, synthetic construct
  misc_feature 1..40: note = Description of Artificial Sequence: primer
  source 1..40: mol_type = other DNA
ttccgggaataccatttttctcagttgatttgtttgtggg

SEQ ID NO: 8 - DNA, 40 bp, synthetic construct
  misc_feature 1..40: note = Description of Artificial Sequence: primer
  source 1..40: mol_type = other DNA
caaatcaactgagaaaaatggtattcccggaaagaactcg

SEQ ID NO: 9 - DNA, 20 bp, synthetic construct
  misc_feature 1..20: note = Description of Artificial Sequence: primer
  source 1..20: mol_type = other DNA
cctggtcttctgtgagtatc

SEQ ID NO: 10 - DNA, 20 bp, synthetic construct
  misc_feature 1..20: note = Description of Artificial Sequence: primer
  source 1..20: mol_type = other DNA
tgggcaggcttgtctgtttg

SEQ ID NO: 11 - DNA, 40 bp, synthetic construct
  misc_feature 1..40: note = Description of Artificial Sequence: primer
  source 1..40: mol_type = other DNA
catagatacaacataaactaggaatgtttccagcggtatg

SEQ ID NO: 12 - DNA, 40 bp, synthetic construct
  misc_feature 1..40: note = Description of Artificial Sequence: primer
  source 1..40: mol_type = other DNA
cataccgctggaaacattcctagtttatgttgtatctatg

SEQ ID NO: 13 - DNA, 19 bp, synthetic construct
  misc_feature 1..19: note = Description of Artificial Sequence: primer
  source 1..19: mol_type = other DNA
ctgactggacttagcgaag

SEQ ID NO: 14 - protein, 571 aa, synthetic construct
  REGION 1..571: note = Description of Artificial Sequence: recombinant peptide
GAPGAPGLQGAPGLQGMPGERGAAGLPGPKGERGDAGPKGADGAPGAPGLQGMPGERGAAGLPGPKGERGDAGPKGADGAPGKDGVRGLAGPIGPPGERGAAGLPGPKGERGDAGPKGADGAPGKDGVRGLAGPIGPPGPAGAPGAPGLQGMPGERGAAGLPGPKGERGDAGPKGADGAPGKDGVRGLAGPPGAPGLQGAPGLQGMPGERGAAGLPGPKGERGDAGPKGADGAPGAPGLQGMPGERGAAGLPGPKGERGDAGPKGADGAPGKDGVRGLAGPIGPPGERGAAGLPGPKGERGDAGPKGADGAPGKDGVRGLAGPIGPPGPAGAPGAPGLQGMPGERGAAGLPGPKGERGDAGPKGADGAPGKDGVRGLAGPPGAPGLQGAPGLQGMPGERGAAGLPGPKGERGDAGPKGADGAPGAPGLQGMPGERGAAGLPGPKGERGDAGPKGADGAPGKDGVRGLAGPIGPPGERGAAGLPGPKGERGDAGPKGADGAPGKDGVRGLAGPIGPPGPAGAPGAPGLQGMPGERGAAGLPGPKGERGDAGPKGADGAPGKDGVRGLAGPPG

SEQ ID NO: 15 - DNA, 5521 bp, synthetic construct
  misc_feature 1..5521: note = Description of Artificial Sequence: plasmid
  source 1..5521: mol_type = other DNA
agatctgcttgcccattcttaatccggctgaattttggtgcgtgatcgcggcccaagtttgcttccagaaagagcttagaataatgctttttacctttgatgaatgctcgcgagtgctcgttttaattaccccatacgcattgttgcagtatgcaagcaccattgcaaatcacgcatggaagaattctgcaaacacgtatagccccgcgttgttgaggaggaggacttagtgtaagaccataaagctgtgtattatggtgagctctgttgtctggtgaccctctgttttggccacgccttggaaaacacactctggcaaatcctcatttttgtgcatgagattcgagccaacagcacaataggacgctcgcggcctattgctccacgaaataattgcgaaatctaaattatgacgcaaggctgagagattctggcacgccgcatttgcggggaaataataatcggggaattttccggggttcgggatggggcttggaaagaaggttcaacacagaccaaaacaacttggcaatgcacgcagacgtttatgcgataccccgagccagcttaggacgagttagatgaagaagagccccgcaaaaagagtttcggcgcgttggacaaacattgatactccacggcaaattaactacagttccgtgtatgcggatagggatatcttcgggagtatcgcaatagaaagcaggcactgtgcagattacgcgacatgatagctttgtatgttctacagactctgccgtaccactctacatataatgtgagagctctgcagcgtcgtaatgaacacttgggttatacaagtttcctaagagccctttgacgttgattgctctggcttccctacgggctctcatgtggttcaagtgactccgcagtggctagcaagcgtgggggtcaattacgtcacttctattcatgtaccccagactcaattgttggcagttatttcagcgagaattaaatgtgcaaattaattctcgctcaaataaattaggccgtgatttaatactcgctgaaacaggatcttgtctggggtacagataacaatcaaataactattatggacgtgcataggaggtggagcccatgacgcaaacggaaatcctctttttattttcgggaagttaggaggataccaaagcgtcgcgctcgctaaagtgatgagaatgtctttagtaagctcaagccatataaagaccctccgcctccacaatttttttatccctcttgacaatattaattccttatgagatttccttcaatttttactgctgttttattcgcagcatcctccgcattagctgctccagtcaacactacaacagaagatgaaacggcacaaattccggctgaagctgtcatcggttactcagatttagaaggggatttcgatgttgctgttttgccattttccaacagcacaaataacgggttattgtttataaatactactattgccagcattgctgctaaagaagaaggggtatctctcgagaaaagagaggctgaagctggagcaccaggtgccccaggcttgcaaggagctcctggcctgcagggtatgccaggagagagaggtgccgctggcttgccaggtccaaagggagagagaggtgatgccggtccaaagggcgctgatggagcaccgggtgctccaggtttgcagggaatgcctggcgaaagaggcgccgccggattgccaggtccaaaaggcgaacgtggagatgctggtcctaagggtgcagatggagctccaggtaaagacggcgttagaggtctggcaggtccaattggacctccaggtgagagaggagctgcaggattgccaggcccaaagggtgaacgtggcgacgccggtccaaagggagcagatggagctccgggtaaagatggagtgagaggactggcaggccctatcggtccaccaggaccagctggtgccccaggcgctcctggtttgcaaggtatgcctggagagagaggtgcagctggactgccaggcccaaaaggtgaaagaggtgatgccggaccaaaaggcgccgatggtgctccaggtaaagatggcgttagaggtcttgctggtccacccggagcccctggcttgcagggcgcaccaggattgcagggtatgccaggcgagagaggagctgcaggtctgcctggtccaaaaggtgaaagaggagatgctggtcctaagggtgctgacggcgcccctggagctccaggattgcagggaatgccaggtgagagaggcgctgccggtttgccaggacctaagggtgaaagaggtgatgctggcccaaaaggtgccgatggagctccaggaaaagatggtgttagaggactggccggtcctatcggccctcctggagaaagaggagctgctggtttgcctggcccaaaaggcgagagaggtgacgctggcccaaaaggagccgacggtgctcctggcaaggacggagtgagaggcctggccggtcctattggtccaccaggacctgctggcgctccaggagctcctggtttgcagggtatgccaggtgaaagaggagccgcaggcctgccaggtcctaagggtgagagaggtgacgccggtcctaaaggcgctgatggagctcctggtaaagatggcgttagaggtttggccggacccccaggtgccccaggtctgcaaggagctccaggtcttcagggtatgccaggcgaaagaggagctgctggtttgccaggcccaaagggtgaaagaggagatgccggcccaaaaggagctgacggtgcaccaggcgctccaggcctgcagggtatgccaggagaaagaggtgctgctggtttgccaggaccaaagggagaaagaggcgacgccggtccaaagggtgcagatggagctcctggcaaagacggagtgagaggcttggcaggtccaatcggaccgccaggcgagagaggtgctgccggcttgccaggtccaaagggtgaaagaggagacgcaggtcctaaaggtgctgacggcgcaccaggaaaagatggtgttagaggtctggctggacctatcggcccaccaggaccagctggtgctccaggtgctcctggccttcagggcatgccaggagaaagaggtgctgccggtctgcctggacctaagggcgaaagaggcgatgcaggtccaaagggtgctgatggagctcctggtaaagatggtgttagaggattggcaggcccacccgggtaatagtctagagtcgactgagtttgtagccttagacatgactgttcctcagttcaagttgggcacttacgagaagaccggtcttgctagattctaatcaagaggatgtcagaatgccatttgcctgagagatgcaggcttcatttttgatacttttttatttgtaacctatatagtataggattttttttgtcattttgtttcttctcgtacgagcttgctcctgatcagcctatctcgcagctgatgaatatcttgtggtaggggtttgggaaaatcattcgagtttgatgtttttcttggtatttcccactcctcttcagagtacagaagattaagtgagaccttcgtttgtgcactagtcccacacaccatagcttcaaaatgtttctactccttttttactcttccagattttctcggactccgcgcatcgccgtaccacttcaaaacacccaagcacagcatactaaattttccctctttcttcctctagggtgtcgttaattacccgtactaaaggtttggaaaagaaaaaagagaccgcctcgtttctttttcttcgtcgaaaaaggcaataaaaatttttatcacgtttctttttcttgaaatttttttttttagtttttttctctttcagtgacctccattgatatttaagttaataaacggtcttcaatttctcaagtttcagtttcatttttcttgttctattacaactttttttacttcttgttcattagaaagaaagcatagcaatctaatctaaggggcggtgttgacaattaatcatcggcatagtatatcggcatagtataatacgacaaggtgaggaactaaaccatggccaagttgaccagtgccgttccggtgctcaccgcgcgcgacgtcgccggagcggtcgagttctggaccgaccggctcgggttctcccgcgacttcgtggaggacgacttcgccggtgtggtccgggacgacgtgaccctgttcatcagcgcggtccaggaccaggtggtgccggacaacaccctggcctgggtgtgggtgcgcggcctggacgagctgtacgccgagtggtcggaggtcgtgtccacgaacttccgggacgcctccgggccggccatgaccgagatcggcgagcagccgtgggggcgggagttcgccctgcgcgacccggccggcaactgcgtgcacttcgtcgccgaggagcaggactgacacgtccgacggcggcccacgggtcccaggcctcggagatccgtcccccttttcctttgtcgatatcatgtaattagttatgtcacgcttacattcacgccctccccccacatccgctctaaccgaaaaggaaggagttagacaacctgaagtctaggtccctatttatttttttatagttatgttagtattaagaacgttatttatatttcaaatttttcttttttttctgtacagacgcgtgtacgcatgtaacattatactgaaaaccttgcttgagaaggttttgggacgctcgaaggctttaatttgcaagctggagaccaacatgtgagcaaaaggccagcaaaaggccaggaaccgtaaaaaggccgcgttgctggcgtttttccataggctccgcccccctgacgagcatcacaaaaatcgacgctcaagtcagaggtggcgaaacccgacaggactataaagataccaggcgtttccccctggaagctccctcgtgcgctctcctgttccgaccctgccgcttaccggatacctgtccgcctttctcccttcgggaagcgtggcgctttctcatagctcacgctgtaggtatctcagttcggtgtaggtcgttcgctccaagctgggctgtgtgcacgaaccccccgttcagcccgaccgctgcgccttatccggtaactatcgtcttgagtccaacccggtaagacacgacttatcgccactggcagcagccactggtaacaggattagcagagcgaggtatgtaggcggtgctacagagttcttgaagtggtggcctaactacggctacactagaagaacagtatttggtatctgcgctctgctgaagccagttaccttcggaaaaagagttggtagctcttgatccggcaaacaaaccaccgctggtagcggtggtttttttgtttgcaagcagcagattacgcgcagaaaaaaaggatctcaagaagatcctttgatcttttctacggggtctgacgctcagtggaacgaaaactcacgttaagggattttggtcatgagatc

SEQ ID NO: 16 - DNA, 1261 bp, synthetic construct
  misc_feature 1..1261: note = Description of Artificial Sequence: recombinant DNA
  source 1..1261: mol_type = other DNA
gcttgcccattcttaatccggctgaattttggtgcgtgatcgcggcccaagtttgcttccagaaagagcttagaataatgctttttacctttgatgaatgctcgcgagtgctcgttttaattaccccatacgcattgttgcagtatgcaagcaccattgcaaatcacgcatggaagaattctgcaaacacgtatagccccgcgttgttgaggaggaggacttagtgtaagaccataaagctgtgtattatggtgagctctgttgtctggtgaccctctgttttggccacgccttggaaaacacactctggcaaatcctcatttttgtgcatgagattcgagccaacagcacaataggacgctcgcggcctattgctccacgaaataattgcgaaatctaaattatgacgcaaggctgagagattctggcacgccgcatttgcggggaaataataatcggggaattttccggggttcgggatggggcttggaaagaaggttcaacacagaccaaaacaacttggcaatgcacgcagacgtttatgcgataccccgagccagcttaggacgagttagatgaagaagagccccgcaaaaagagtttcggcgcgttggacaaacattgatactccacggcaaattaactacagttccgtgtatgcggatagggatatcttcgggagtatcgcaatagaaagcaggcactgtgcagattacgcgacatgatagctttgtatgttctacagactctgccgtaccactctacatataatgtgagagctctgcagcgtcgtaatgaacacttgggttatacaagtttcctaagagccctttgacgttgattgctctggcttccctacgggctctcatgtggttcaagtgactccgcagtggctagcaagcgtgggggtcaattacgtcacttctattcatgtaccccagactcaattgttggcagttatttcagcgagaattaaatgtgcaaattaattctcgctcaaataaattaggccgtgatttaatactcgctgaaacaggatcttgtctggggtacagataacaatcaaataactattatggacgtgcataggaggtggagcccatgacgcaaacggaaatcctctttttattttcgggaagttaggaggataccaaagcgtcgcgctcgctaaagtgatgagaatgtctttagtaagctcaagccatataaagaccctccgcctccacaatttttttatccctcttgacaatattaattcctt

SEQ ID NO: 17 - DNA, 267 bp, synthetic construct
  misc_feature 1..267: note = Description of Artificial Sequence: recombinant DNA
  source 1..267: mol_type = other DNA
atgagatttccttcaatttttactgctgttttattcgcagcatcctccgcattagctgctccagtcaacactacaacagaagatgaaacggcacaaattccggctgaagctgtcatcggttactcagatttagaaggggatttcgatgttgctgttttgccattttccaacagcacaaataacgggttattgtttataaatactactattgccagcattgctgctaaagaagaaggggtatctctcgagaaaagagaggctgaagct

SEQ ID NO: 18 - DNA, 1713 bp, synthetic construct
  misc_feature 1..1713: note = Description of Artificial Sequence: recombinant DNA
  source 1..1713: mol_type = other DNA
ggagcaccaggtgccccaggcttgcaaggagctcctggcctgcagggtatgccaggagagagaggtgccgctggcttgccaggtccaaagggagagagaggtgatgccggtccaaagggcgctgatggagcaccgggtgctccaggtttgcagggaatgcctggcgaaagaggcgccgccggattgccaggtccaaaaggcgaacgtggagatgctggtcctaagggtgcagatggagctccaggtaaagacggcgttagaggtctggcaggtccaattggacctccaggtgagagaggagctgcaggattgccaggcccaaagggtgaacgtggcgacgccggtccaaagggagcagatggagctccgggtaaagatggagtgagaggactggcaggccctatcggtccaccaggaccagctggtgccccaggcgctcctggtttgcaaggtatgcctggagagagaggtgcagctggactgccaggcccaaaaggtgaaagaggtgatgccggaccaaaaggcgccgatggtgctccaggtaaagatggcgttagaggtcttgctggtccacccggagcccctggcttgcagggcgcaccaggattgcagggtatgccaggcgagagaggagctgcaggtctgcctggtccaaaaggtgaaagaggagatgctggtcctaagggtgctgacggcgcccctggagctccaggattgcagggaatgccaggtgagagaggcgctgccggtttgccaggacctaagggtgaaagaggtgatgctggcccaaaaggtgccgatggagctccaggaaaagatggtgttagaggactggccggtcctatcggccctcctggagaaagaggagctgctggtttgcctggcccaaaaggcgagagaggtgacgctggcccaaaaggagccgacggtgctcctggcaaggacggagtgagaggcctggccggtcctattggtccaccaggacctgctggcgctccaggagctcctggtttgcagggtatgccaggtgaaagaggagccgcaggcctgccaggtcctaagggtgagagaggtgacgccggtcctaaaggcgctgatggagctcctggtaaagatggcgttagaggtttggccggacccccaggtgccccaggtctgcaaggagctccaggtcttcagggtatgccaggcgaaagaggagctgctggtttgccaggcccaaagggtgaaagaggagatgccggcccaaaaggagctgacggtgcaccaggcgctccaggcctgcagggtatgccaggagaaagaggtgctgctggtttgccaggaccaaagggagaaagaggcgacgccggtccaaagggtgcagatggagctcctggcaaagacggagtgagaggcttggcaggtccaatcggaccgccaggcgagagaggtgctgccggcttgccaggtccaaagggtgaaagaggagacgcaggtcctaaaggtgctgacggcgcaccaggaaaagatggtgttagaggtctggctggacctatcggcccaccaggaccagctggtgctccaggtgctcctggccttcagggcatgccaggagaaagaggtgctgccggtctgcctggacctaagggcgaaagaggcgatgcaggtccaaagggtgctgatggagctcctggtaaagatggtgttagaggattggcaggcccacccggg

SEQ ID NO: 19 - DNA, 5269 bp, synthetic construct
  misc_feature 1..5269: note = Description of Artificial Sequence: plasmid
  source 1..5269: mol_type = other DNA
agatctaacatccaaagacgaaaggttgaatgaaacctttttgccatccgacatccacaggtccattctcacacataagtgccaaacgcaacaggaggggatacactagcagcagaccgttgcaaacgcaggacctccactcctcttctcctcaacacccacttttgccatcgaaaaaccagcccagttattgggcttgattggagctcgctcattccaattccttctattaggctactaacaccatgactttattagcctgtctatcctggcccccctggcgaggttcatgtttgtttatttccgaatgcaacaagctccgcattacacccgaacatcactccagatgagggctttctgagtgtggggtcaaatagtttcatgttccccaaatggcccaaaactgacagtttaaacgctgtcttggaacctaatatgacaaaagcgtgatctcatccaagatgaactaagtttggttcgttgaaatgctaacggccagttggtcaaaaagaaacttccaaaagtcggcataccgtttgtcttgtttggtattgattgacgaatgctcaaaaataatctcattaatgcttagcgcagtctctctatcgcttctgaaccccggtgcacctgtgccgaaacgcaaatggggaaacacccgctttttggatgattatgcattgtctccacattgtatgcttccaagattctggtgggaatactgctgatagcctaacgttcatgatcaaaatttaactgttctaacccctacttgacagcaatatataaacagaaggaagctgccctgtcttaaacctttttttttatcatcattattagcttactttcataattgcgactggttccaattgacaagcttttgattttaacgacttttaacgacaacttgagaagatcaaaaaacaactaattattcgaagaatccaaacgatgagatttccttcaatttttactgcagttttattcgcagcatcctccgcattagctgctccagtcaacactacaacagaagatgaaacggcacaaattccggctgaagctgtcatcggttactcagatttagaaggggatttcgatgttgctgttttgccattttccaacagcacaaataacgggttattgtttataaatactactattgccagcattgctgctaaagaagaaggggtatctctcgagaaaagagaggctgaagctggagctccaggtgctccaggccttcagggtgctccaggtttgcagggtatgccaggagagagaggagctgccggtttgcctggcccaaagggtgagagaggtgacgctggtcctaaaggtgctgacggagctccaggagctcctggactgcaaggcatgcctggtgaaagaggtgcagctggcctgccaggaccaaaaggagaaagaggcgatgcaggcccaaagggagcagatggtgccccaggtaaagacggtgttagaggcttggctggacctatcggacctccaggtgaaagaggtgcagctggcctgccaggaccaaaaggagaaagaggcgatgcaggcccaaagggagcagatggtgccccaggtaaagacggtgttagaggcttggctggacctatcggaccacctggtccagctggagcccctggtgctccaggtttgcagggtatgccaggagagagaggagctgccggtttgcctggtccaaagggcgaaagaggtgatgccggaccgaaaggcgctgatggcgccccaggcaaggatggcgtgagaggtctggccggtccacccggtgctccaggccttcagggtgctccaggtttgcagggtatgccaggagagagaggagctgccggtttgcctggcccaaagggtgagagaggtgacgctggtcctaaaggtgctgacggagctccaggagctcctggactgcaaggcatgcctggtgaaagaggtgcagctggcctgccaggaccaaaaggagaaagaggcgatgcaggcccaaagggagcagatggtgccccaggtaaagacggtgttagaggcttggctggacctatcggacctccaggtgaaagaggtgcagctggcctgccaggaccaaaaggagaaagaggcgatgcaggcccaaagggagcagatggtgccccaggtaaagacggtgttagaggcttggctggacctatcggaccacctggtccagctggagcccctggtgctccaggtttgcagggtatgccaggagagagaggagctgccggtttgcctggtccaaagggcgaaagaggtgatgccggaccgaaaggcgctgatggcgccccaggcaaggatggcgtgagaggtctggccggtccacccggtgctccaggccttcagggtgctccaggtttgcagggtatgccaggagagagaggagctgccggtttgcctggcccaaagggtgagagaggtgacgctggtcctaaaggtgctgacggagctccaggagctcctggactgcaaggcatgcctggtgaaagaggtgcagctggcctgccaggaccaaaaggagaaagaggcgatgcaggcccaaagggagcagatggtgccccaggtaaagacggtgttagaggcttggctggacctatcggacctccaggtgaaagaggtgcagctggcctgccaggaccaaaaggagaaagaggcgatgcaggcccaaagggagcagatggtgccccaggtaaagacggtgttagaggcttggctggacctatcggaccacctggtccagctggagcccctggtgctccaggtttgcagggtatgccaggagagagaggagctgccggtttgcctggtccaaagggcgaaagaggtgatgccggaccgaaaggcgctgatggcgccccaggcaaggatggcgtgagaggtctggccggtccacccgggtaagcggccgccagctttctagaacaaaaactcatctcagaagaggatctgaatagcgccgtcgaccatcatcatcatcatcattgagtttgtagccttagacatgactgttcctcagttcaagttgggcacttacgagaagaccggtcttgctagattctaatcaagaggatgtcagaatgccatttgcctgagagatgcaggcttcatttttgatacttttttatttgtaacctatatagtataggattttttttgtcattttgtttcttctcgtacgagcttgctcctgatcagcctatctcgcagctgatgaatatcttgtggtaggggtttgggaaaatcattcgagtttgatgtttttcttggtatttcccactcctcttcagagtacagaagattaagtgagaccttcgtttgtgcggatcccccacacaccatagcttcaaaatgtttctactccttttttactcttccagattttctcggactccgcgcatcgccgtaccacttcaaaacacccaagcacagcatactaaatttcccctctttcttcctctagggtgtcgttaattacccgtactaaaggtttggaaaagaaaaaagagaccgcctcgtttctttttcttcgtcgaaaaaggcaataaaaatttttatcacgtttctttttcttgaaaatttttttttttgatttttttctctttcgatgacctcccattgatatttaagttaataaacggtcttcaatttctcaagtttcagtttcatttttcttgttctattacaactttttttacttcttgctcattagaaagaaagcatagcaatctaatctaagggcggtgttgacaattaatcatcggcatagtatatcggcatagtataatacgacaaggtgaggaactaaaccatggccaagttgaccagtgccgttccggtgctcaccgcgcgcgacgtcgccggagcggtcgagttctggaccgaccggctcgggttctcccgggacttcgtggaggacgacttcgccggtgtggtccgggacgacgtgaccctgttcatcagcgcggtccaggaccaggtggtgccggacaacaccctggcctgggtgtgggtgcgcggcctggacgagctgtacgccgagtggtcggaggtcgtgtccacgaacttccgggacgcctccgggccggccatgaccgagatcggcgagcagccgtgggggcgggagttcgccctgcgcgacccggccggcaactgcgtgcacttcgtggccgaggagcaggactgacacgtccgacgcggcccgacgggtccgaggcctcggagatccgtcccccttttcctttgtcgatatcatgtaattagttatgtcacgcttacattcacgccctccccccacatccgctctaaccgaaaaggaaggagttagacaacctgaagtctaggtccctatttatttttttatagttatgttagtattaagaacgttatttatatttcaaatttttcttttttttctgtacagacgcgtgtacgcatgtaacattatactgaaaaccttgcttgagaaggttttgggacgctcgaaggctttaatttgcaagctggagaccaacatgtgagcaaaaggccagcaaaaggccaggaaccgtaaaaaggccgcgttgctggcgtttttccataggctccgcccccctgacgagcatcacaaaaatcgacgctcaagtcagaggtggcgaaacccgacaggactataaagataccaggcgtttccccctggaagctccctcgtgcgctctcctgttccgaccctgccgcttaccggatacctgtccgcctttctcccttcgggaagcgtggcgctttctcatagctcacgctgtaggtatctcagttcggtgtaggtcgttcgctccaagctgggctgtgtgcacgaaccccccgttcagcccgaccgctgcgccttatccggtaactatcgtcttgagtccaacccggtaagacacgacttatcgccactggcagcagccactggtaacaggattagcagagcgaggtatgtaggcggtgctacagagttcttgaagtggtggcctaactacggctacactagaagaacagtatttggtatctgcgctctgctgaagccagttaccttcggaaaaagagttggtagctcttgatccggcaaacaaaccaccgctggtagcggtggtttttttgtttgcaagcagcagattacgcgcagaaaaaaaggatctcaagaagatcctttgatcttttctacggggtctgacgctcagtggaacgaaaactcacgttaagggattttggtcatgagatc